European Patent Application EP 4 775 676 A1, published July 15, 2026. Title: Phosphodiesterase and use thereof. Applicant: 天野エンザイム株式会社. The sequence listing filed with the application follows.

SEQUENCE LISTING (6 sequences)

SEQ ID NO: 1 - protein, 318 aa, Leptographium procerum
  source 1..318: note = phosphodiesterase of the present invention (without signal peptide)
WGTLGHATVAYIAQDFLTSDAKAWAQDVLSDTSTSYLASVASWADSYRATAAGKWSAPFHFIDAEDDPPSSCSVDYDRDCGSSGCSVSAIANYTRRVGSSELSAANVNQAFKFLVHLVGDITQPLHDEALDKGGNEITVTFDGYDSDNLHSDWDTYIPQKLTGGSSLAVARQWATNLTADIKTGTYKSAKAAWIDGDDITEAVATATRWASDANALVCSVVMPNGVAALQSGDLYPTYYDSVVPTVELQIAKGGYRLANWLNLIYESDIAATKRRRSPAPAPEPQPDLSGADLLPPPRPLSKAKLARAAMNGECCHAH

SEQ ID NO: 2 - protein, 338 aa, Leptographium procerum
  source 1..338: note = phosphodiesterase of the present invention
MHSPAVVLLSLAATLRGAQAWGTLGHATVAYIAQDFLTSDAKAWAQDVLSDTSTSYLASVASWADSYRATAAGKWSAPFHFIDAEDDPPSSCSVDYDRDCGSSGCSVSAIANYTRRVGSSELSAANVNQAFKFLVHLVGDITQPLHDEALDKGGNEITVTFDGYDSDNLHSDWDTYIPQKLTGGSSLAVARQWATNLTADIKTGTYKSAKAAWIDGDDITEAVATATRWASDANALVCSVVMPNGVAALQSGDLYPTYYDSVVPTVELQIAKGGYRLANWLNLIYESDIAATKRRRSPAPAPEPQPDLSGADLLPPPRPLSKAKLARAAMNGECCHAH

SEQ ID NO: 3 - DNA, 957 bp, Leptographium procerum
  source 1..957: mol_type = genomic DNA; note = nucleotide sequence encoding phosphodiesterase of the present invention (without signal peptide)
tggggcactctgggccacgccacggtcgcgtatatcgcgcaggactttctgacgagcgacgccaaggcctgggcccaggacgtgctctcagacacgtcgacatcgtacctggccagcgtggcgtcgtgggcggactcgtatcgggccacggcagccggcaagtggtctgcgcccttccacttcatcgacgccgaggacgacccgccgtcgagctgcagcgtcgactacgaccgcgactgcggcagctccggctgctctgtcagcgccatcgccaactacacgcgccgcgtcggcagcagcgagctgtcggccgccaacgtcaaccaggccttcaagttcctggtccacctcgtcggcgacatcacgcagccgctgcacgacgaggccctcgacaagggcggcaacgagatcaccgtcacctttgacggctacgactccgacaacctgcactccgactgggacacgtacatcccccagaagctgaccggcggcagcagcctcgccgtcgcccgccagtgggccaccaacctcaccgccgacatcaagaccggcacctacaagtccgccaaggccgcctggatcgacggcgacgacatcaccgaggccgtcgccaccgccactcgctgggcctcggacgcaaacgccctcgtctgctctgtcgtcatgcccaacggcgttgccgccctgcagtccggcgacctctacccgacctactacgacagcgtcgtgcccaccgtcgagctgcagattgcaaagggcggctaccgcctcgccaactggctcaacctcatctacgagtccgacatcgccgccacaaagcgccgccgctctcctgctcccgccccggagccccagcccgacctctcgggcgccgacctgctgccacccccccggccgctcagcaaggccaagcttgcacgtgccgctatgaacggcgagtgctgccatgcgcattaa

SEQ ID NO: 4 - DNA, 1017 bp, Leptographium procerum
  source 1..1017: mol_type = genomic DNA; note = nucleotide sequence encoding phosphodiesterase of the present invention
atgcactctcccgccgtcgtcctcctcagcctcgcggccaccctgagaggcgcgcaggcctggggcactctgggccacgccacggtcgcgtatatcgcgcaggactttctgacgagcgacgccaaggcctgggcccaggacgtgctctcagacacgtcgacatcgtacctggccagcgtggcgtcgtgggcggactcgtatcgggccacggcagccggcaagtggtctgcgcccttccacttcatcgacgccgaggacgacccgccgtcgagctgcagcgtcgactacgaccgcgactgcggcagctccggctgctctgtcagcgccatcgccaactacacgcgccgcgtcggcagcagcgagctgtcggccgccaacgtcaaccaggccttcaagttcctggtccacctcgtcggcgacatcacgcagccgctgcacgacgaggccctcgacaagggcggcaacgagatcaccgtcacctttgacggctacgactccgacaacctgcactccgactgggacacgtacatcccccagaagctgaccggcggcagcagcctcgccgtcgcccgccagtgggccaccaacctcaccgccgacatcaagaccggcacctacaagtccgccaaggccgcctggatcgacggcgacgacatcaccgaggccgtcgccaccgccactcgctgggcctcggacgcaaacgccctcgtctgctctgtcgtcatgcccaacggcgttgccgccctgcagtccggcgacctctacccgacctactacgacagcgtcgtgcccaccgtcgagctgcagattgcaaagggcggctaccgcctcgccaactggctcaacctcatctacgagtccgacatcgccgccacaaagcgccgccgctctcctgctcccgccccggagccccagcccgacctctcgggcgccgacctgctgccacccccccggccgctcagcaaggccaagcttgcacgtgccgctatgaacggcgagtgctgccatgcgcattaa

SEQ ID NO: 5 - protein, 7 aa, Leptographium procerum
  source 1..7: note = amino acid sequecen of active senter of phosphodiesterase of the present invention
DSYRATA

SEQ ID NO: 6 - DNA, 21 bp, Leptographium procerum
  source 1..21: mol_type = genomic DNA; note = nucleotide sequence encoding the active center of phosphodiesterase of the present invention
gactcgtatcgggccacggca